European Patent Specification EP 3 471 765 B1, published April 24, 2024. Title: HIV Vaccine Formulation. Applicant: Janssen Vaccines & Prevention B.V. The sequence listing filed with the application follows.

SEQUENCE LISTING (14 sequences)

SEQ ID NO: 1 - protein, 679 aa, Artificial Sequence
  HIV clade C gp140 protein
AENLWVGNMWVTVYYGVPVWTDAKTTLFCASDTKAYDREVHNVWATHACVPTDPNPQEIVLENVTENFNMWKNDMVDQMHEDIISLWDQSLKPCVKLTPLCVTLHCTNATFKNNVTNDMNKEIRNCSFNTTTEIRDKKQQGYALFYRPDIVLLKENRNNSNNSEYILINCNASTITQACPKVNFDPIPIHYCAPAGYAILKCNNKTFSGKGPCNNVSTVQCTHGIKPVVSTQLLLNGSLAEKEIIIRSENLTDNVKTIIVHLNKSVEIVCTRPNNNTRKSMRIGPGQTFYATGDIIGDIRQAYCNISGSKWNETLKRVKEKLQENYNNNKTIKFAPSSGGDLEITTHSFNCRGEFFYCNTTRLFNNNATEDETITLPCRIKQIINMWQGVGRAMYAPPIAGNITCKSNITGLLLVRDGGEDNKTEEIFRPGGGNMKDNWRSELYKYKVIELKPLGIAPTGAKERVVEREERAVGIGAVFLGFLGAAGSTMGAASLTLTVQARQLLSSIVQQQSNLLRAIEAQQHMLQLTVWGIKQLQTRVLAIERYLKDQQLLGIWGCSGKLICTTNVPWNSSWSNKSQTDIWNNMTWMEWDREISNYTDTIYRLLEDSQTQQEKNEKDLLALDSWKNLWSWFDISNWLWYIKSRIEGRGSGGYIPEAPRDGQAYVRKDGEWVLLSTFL

SEQ ID NO: 2 - protein, 695 aa, Artificial Sequence
  HIV mosaic gp140 protein
AGKLWVTVYYGVPVWKEATTTLFCASDAKAYDTEVHNVWATHACVPTDPNPQEVVLENVTENFNMWKNNMVEQMHEDIISLWDQSLKPCVKLTPLCVTLNCTDDVRNVTNNATNTNSSWGEPMEKGEIKNCSFNITTSIRNKVQKQYALFYKLDVVPIDNDSNNTNYRLISCNTSVITQACPKVSFEPIPIHYCAPAGFAILKCNDKKFNGTGPCTNVSTVQCTHGIRPVVSTQLLLNGSLAEEEVVIRSENFTNNAKTIMVQLNVSVEINCTRPNNNTRKSIHIGPGRAFYTAGDIIGDIRQAHCNISRANWNNTLRQIVEKLGKQFGNNKTIVFNHSSGGDPEIVMHSFNCGGEFFYCNSTKLFNSTWTWNNSTWNNTKRSNDTEEHITLPCRIKQIINMWQEVGKAMYAPPIRGQIRCSSNITGLLLTRDGGNDTSGTEIFRPGGGDMRDNWRSELYKYKVVKIEPLGVAPTKAKERVVQREERAVGIGAVFLGFLGAAGSTMGAASMTLTVQARLLLSGIVQQQNNLLRAIEAQQHLLQLTVWGIKQLQARVLAVERYLKDQQLLGIWGCSGKLICTTTVPWNASWSNKSLDKIWNNMTWMEWEREINNYTSLIYTLIEESQNQQEKNEQELLELDKWASLWNWFDISNWLWYIKSRIEGRGSGGYIPEAPRDGQAYVRKDGEWVLLSTFL

SEQ ID NO: 3 - protein, 660 aa, Artificial Sequence
  Mos1Env mosaic HIV antigen
MRVTGIRKNYQHLWRWGTMLLGILMICSAAGKLWVTVYYGVPVWKEATTTLFCASDAKAYDTEVHNVWATHACVPTDPNPQEVVLENVTENFNMWKNNMVEQMHEDIISLWDQSLKPCVKLTPLCVTLNCTDDVRNVTNNATNTNSSWGEPMEKGEIKNCSFNITTSIRNKVQKQYALFYKLDVVPIDNDSNNTNYRLISCNTSVITQACPKVSFEPIPIHYCAPAGFAILKCNDKKFNGTGPCTNVSTVQCTHGIRPVVSTQLLLNGSLAEEEVVIRSENFTNNAKTIMVQLNVSVEINCTRPNNNTRKSIHIGPGRAFYTAGDIIGDIRQAHCNISRANWNNTLRQIVEKLGKQFGNNKTIVFNHSSGGDPEIVMHSFNCGGEFFYCNSTKLFNSTWTWNNSTWNNTKRSNDTEEHITLPCRIKQIINMWQEVGKAMYAPPIRGQIRCSSNITGLLLTRDGGNDTSGTEIFRPGGGDMRDNWRSELYKYKVVKIEPLGVAPTKAKRRVVQSEKSAVGIGAVFLGFLGAAGSTMGAASMTLTVQARLLLSGIVQQQNNLLRAIEAQQHLLQLTVWGIKQLQARVLAVERYLKDQQLLGIWGCSGKLICTTTVPWNASWSNKSLDKIWNNMTWMEWEREINNYTSLIYTLIEESQNQQEK

SEQ ID NO: 4 - protein, 684 aa, Artificial Sequence
  Mos2Env mosaic HIV antigen
MRVRGIQRNWPQWWIWGILGFWMIIICRVMGNLWVTVYYGVPVWKEAKTTLFCASDAKAYEKEVHNVWATHACVPTDPNPQEMVLENVTENFNMWKNDMVDQMHEDIIRLWDQSLKPCVKLTPLCVTLECRNVRNVSSNGTYNIIHNETYKEMKNCSFNATTVVEDRKQKVHALFYRLDIVPLDENNSSEKSSENSSEYYRLINCNTSAITQACPKVSFDPIPIHYCAPAGYAILKCNNKTFNGTGPCNNVSTVQCTHGIKPVVSTQLLLNGSLAEEEIIIRSENLTNNAKTIIVHLNETVNITCTRPNNNTRKSIRIGPGQTFYATGDIIGDIRQAHCNLSRDGWNKTLQGVKKKLAEHFPNKTINFTSSSGGDLEITTHSFNCRGEFFYCNTSGLFNGTYMPNGTNSNSSSNITLPCRIKQIINMWQEVGRAMYAPPIAGNITCRSNITGLLLTRDGGSNNGVPNDTETFRPGGGDMRNNWRSELYKYKVVEVKPLGVAPTEAKRRVVESEKSAVGIGAVFLGILGAAGSTMGAASITLTVQARQLLSGIVQQQSNLLRAIEAQQHMLQLTVWGIKQLQTRVLAIERYLQDQQLLGLWGCSGKLICTTAVPWNTSWSNKSQTDIWDNMTWMQWDKEIGNYTGEIYRLLEESQNQQEKNEKDLLALDSWKNLWNWFDITNWLW

SEQ ID NO: 5 - protein, 840 aa, Artificial Sequence
  Mos1Pol mosaic HIV antigen
MAPISPIETVPVKLKPGMDGPRVKQWPLTEEKIKALTAICEEMEKEGKITKIGPENPYNTPVFAIKKKDSTKWRKLVDFRELNKRTQDFWEVQLGIPHPAGLKKKKSVTVLAVGDAYFSVPLDEGFRKYTAFTIPSTNNETPGIRYQYNVLPQGWKGSPAIFQCSMTRILEPFRAKNPEIVIYQYMAALYVGSDLEIGQHRAKIEELREHLLKWGFTTPDKKHQKEPPFLWMGYELHPDKWTVQPIQLPEKDSWTVNDIQKLVGKLNWASQIYPGIKVRQLCKLLRGAKALTDIVPLTEEAELELAENREILKEPVHGVYYDPSKDLIAEIQKQGHDQWTYQIYQEPFKNLKTGKYAKMRTAHTNDVKQLTEAVQKIAMESIVIWGKTPKFRLPIQKETWETWWTDYWQATWIPEWEFVNTPPLVKLWYQLEKDPIAGVETFYVAGAANRETKLGKAGYVTDRGRQKIVSLTETTNQKTALQAIYLALQDSGSEVNIVTASQYALGIIQAQPDKSESELVNQIIEQLIKKERVYLSWVPAHKGIGGNEQVDKLVSSGIRKVLFLDGIDKAQEEHEKYHSNWRAMASDFNLPPVVAKEIVASCDQCQLKGEAMHGQVDCSPGIWQLACTHLEGKIILVAVHVASGYIEAEVIPAETGQETAYFILKLAGRWPVKVIHTANGSNFTSAAVKAACWWAGIQQEFGIPYNPQSQGVVASMNKELKKIIGQVRDQAEHLKTAVQMAVFIHNFKRKGGIGGYSAGERIIDIIATDIQTKELQKQIIKIQNFRVYYRDSRDPIWKGPAKLLWKGEGAVVIQDNSDIKVVPRRKVKIIKDYGKQMAGA

SEQ ID NO: 6 - protein, 850 aa, Artificial Sequence
  Mos2Pol mosaic HIV antigen
MAPISPIETVPVKLKPGMDGPKVKQWPLTEEKIKALVEICTEMEKEGKISKIGPENPYNTPIFAIKKKDSTKWRKLVDFRELNKRTQDFWEVQLGIPHPAGLKKKKSVTVLAVGDAYFSVPLDEDFRKYTAFTIPSINNETPGIRYQYNVLPQGWKGSPAIFQSSMTKILEPFRKQNPDIVIYQYMAALYVGSDLEIGQHRTKIEELRQHLLRWGFTTPDKKHQKEPPFLWMGYELHPDKWTVQPIVLPEKDSWTVNDIQKLVGKLNWASQIYAGIKVKQLCKLLRGTKALTEVVPLTEEAELELAENREILKEPVHGVYYDPSKDLIAEIQKQGQGQWTYQIYQEPFKNLKTGKYARMRGAHTNDVKQLTEAVQKIATESIVIWGKTPKFKLPIQKETWEAWWTEYWQATWIPEWEFVNTPPLVKLWYQLEKEPIVGAETFYVAGAANRETKLGKAGYVTDRGRQKVVSLTDTTNQKTALQAIHLALQDSGLEVNIVTASQYALGIIQAQPDKSESELVSQIIEQLIKKEKVYLAWVPAHKGIGGNEQVDKLVSRGIRKVLFLDGIDKAQEEHEKYHSNWRAMASEFNLPPIVAKEIVASCDKCQLKGEAIHGQVDCSPGIWQLACTHLEGKVILVAVHVASGYIEAEVIPAETGQETAYFLLKLAGRWPVKTIHTANGSNFTSATVKAACWWAGIKQEFGIPYNPQSQGVVASINKELKKIIGQVRDQAEHLKTAVQMAVFIHNFKRKGGIGEYSAGERIVDIIASDIQTKELQKQITKIQNFRVYYRDSRDPLWKGPAKLLWKGEGAVVIQDNSDIKVVPRRKAKIIRDYGKQMAGDDCVASRQDED

SEQ ID NO: 7 - protein, 500 aa, Artificial Sequence
  Mos1Gag mosaic HIV antigen
MGARASVLSGGELDRWEKIRLRPGGKKKYRLKHIVWASRELERFAVNPGLLETSEGCRQILGQLQPSLQTGSEELRSLYNTVATLYCVHQRIEIKDTKEALEKIEEEQNKSKKKAQQAAADTGNSSQVSQNYPIVQNIQGQMVHQAISPRTLNAWVKVVEEKAFSPEVIPMFSALSEGATPQDLNTMLNTVGGHQAAMQMLKETINEEAAEWDRVHPVHAGPIAPGQMREPRGSDIAGTTSTLQEQIGWMTNNPPIPVGEIYKRWIILGLNKIVRMYSPVSILDIRQGPKEPFRDYVDRFYKTLRAEQASQDVKNWMTETLLVQNANPDCKTILKALGPAATLEEMMTACQGVGGPGHKARVLAEAMSQVTNSATIMMQRGNFRNQRKTVKCFNCGKEGHIAKNCRAPRKKGCWKCGKEGHQMKDCTERQANFLGKIWPSNKGRPGNFLQNRPEPTAPPEESFRFGEETTTPSQKQEPIDKEMYPLASLKSLFGNDPSSQ

SEQ ID NO: 8 - protein, 491 aa, Artificial Sequence
  Mos2Gag mosaic HIV antigen
MGARASILRGGKLDKWEKIRLRPGGKKHYMLKHLVWASRELERFALNPGLLETSEGCKQIIKQLQPALQTGTEELRSLFNTVATLYCVHAEIEVRDTKEALDKIEEEQNKSQQKTQQAKEADGKVSQNYPIVQNLQGQMVHQPISPRTLNAWVKVIEEKAFSPEVIPMFTALSEGATPQDLNTMLNTVGGHQAAMQMLKDTINEEAAEWDRLHPVHAGPVAPGQMREPRGSDIAGTTSNLQEQIAWMTSNPPIPVGDIYKRWIILGLNKIVRMYSPTSILDIKQGPKEPFRDYVDRFFKTLRAEQATQDVKNWMTDTLLVQNANPDCKTILRALGPGATLEEMMTACQGVGGPSHKARVLAEAMSQTNSTILMQRSNFKGSKRIVKCFNCGKEGHIARNCRAPRKKGCWKCGKEGHQMKDCTERQANFLGKIWPSHKGRPGNFLQSRPEPTAPPAESFRFEETTPAPKQEPKDREPLTSLRSLFGSDPLSQ

SEQ ID NO: 9 - protein, 1350 aa, Artificial Sequence
  Mos1GagPol mosaic HIV antigen
MGARASVLSGGELDRWEKIRLRPGGKKKYRLKHIVWASRELERFAVNPGLLETSEGCRQILGQLQPSLQTGSEELRSLYNTVATLYCVHQRIEIKDTKEALEKIEEEQNKSKKKAQQAAADTGNSSQVSQNYPIVQNIQGQMVHQAISPRTLNAWVKVVEEKAFSPEVIPMFSALSEGATPQDLNTMLNTVGGHQAAMQMLKETINEEAAEWDRVHPVHAGPIAPGQMREPRGSDIAGTTSTLQEQIGWMTNNPPIPVGEIYKRWIILGLNKIVRMYSPVSILDIRQGPKEPFRDYVDRFYKTLRAEQASQDVKNWMTETLLVQNANPDCKTILKALGPAATLEEMMTACQGVGGPGHKARVLAEAMSQVTNSATIMMQRGNFRNQRKTVKCFNCGKEGHIAKNCRAPRKKGCWKCGKEGHQMKDCTERQANFLGKIWPSNKGRPGNFLQNRPEPTAPPEESFRFGEETTTPSQKQEPIDKEMYPLASLKSLFGNDPSSQMAPISPIETVPVKLKPGMDGPRVKQWPLTEEKIKALTAICEEMEKEGKITKIGPENPYNTPVFAIKKKDSTKWRKLVDFRELNKRTQDFWEVQLGIPHPAGLKKKKSVTVLAVGDAYFSVPLDEGFRKYTAFTIPSTNNETPGIRYQYNVLPQGWKGSPAIFQCSMTRILEPFRAKNPEIVIYQYMAALYVGSDLEIGQHRAKIEELREHLLKWGFTTPDKKHQKEPPFLWMGYELHPDKWTVQPIQLPEKDSWTVNDIQKLVGKLNWASQIYPGIKVRQLCKLLRGAKALTDIVPLTEEAELELAENREILKEPVHGVYYDPSKDLIAEIQKQGHDQWTYQIYQEPFKNLKTGKYAKMRTAHTNDVKQLTEAVQKIAMESIVIWGKTPKFRLPIQKETWETWWTDYWQATWIPEWEFVNTPPLVKLWYQLEKDPIAGVETFYVAGAANRETKLGKAGYVTDRGRQKIVSLTETTNQKTALQAIYLALQDSGSEVNIVTASQYALGIIQAQPDKSESELVNQIIEQLIKKERVYLSWVPAHKGIGGNEQVDKLVSSGIRKVLFLDGIDKAQEEHEKYHSNWRAMASDFNLPPVVAKEIVASCDQCQLKGEAMHGQVDCSPGIWQLACTHLEGKIILVAVHVASGYIEAEVIPAETGQETAYFILKLAGRWPVKVIHTANGSNFTSAAVKAACWWAGIQQEFGIPYNPQSQGVVASMNKELKKIIGQVRDQAEHLKTAVQMAVFIHNFKRKGGIGGYSAGERIIDIIATDIQTKELQKQIIKIQNFRVYYRDSRDPIWKGPAKLLWKGEGAVVIQDNSDIKVVPRRKVKIIKDYGKQMAGADCVAGRQDED

SEQ ID NO: 10 - protein, 1341 aa, Artificial Sequence
  Mos2GagPol mosaic HIV antigen
MGARASILRGGKLDKWEKIRLRPGGKKHYMLKHLVWASRELERFALNPGLLETSEGCKQIIKQLQPALQTGTEELRSLFNTVATLYCVHAEIEVRDTKEALDKIEEEQNKSQQKTQQAKEADGKVSQNYPIVQNLQGQMVHQPISPRTLNAWVKVIEEKAFSPEVIPMFTALSEGATPQDLNTMLNTVGGHQAAMQMLKDTINEEAAEWDRLHPVHAGPVAPGQMREPRGSDIAGTTSNLQEQIAWMTSNPPIPVGDIYKRWIILGLNKIVRMYSPTSILDIKQGPKEPFRDYVDRFFKTLRAEQATQDVKNWMTDTLLVQNANPDCKTILRALGPGATLEEMMTACQGVGGPSHKARVLAEAMSQTNSTILMQRSNFKGSKRIVKCFNCGKEGHIARNCRAPRKKGCWKCGKEGHQMKDCTERQANFLGKIWPSHKGRPGNFLQSRPEPTAPPAESFRFEETTPAPKQEPKDREPLTSLRSLFGSDPLSQMAPISPIETVPVKLKPGMDGPKVKQWPLTEEKIKALVEICTEMEKEGKISKIGPENPYNTPIFAIKKKDSTKWRKLVDFRELNKRTQDFWEVQLGIPHPAGLKKKKSVTVLAVGDAYFSVPLDEDFRKYTAFTIPSINNETPGIRYQYNVLPQGWKGSPAIFQSSMTKILEPFRKQNPDIVIYQYMAALYVGSDLEIGQHRTKIEELRQHLLRWGFTTPDKKHQKEPPFLWMGYELHPDKWTVQPIVLPEKDSWTVNDIQKLVGKLNWASQIYAGIKVKQLCKLLRGTKALTEVVPLTEEAELELAENREILKEPVHGVYYDPSKDLIAEIQKQGQGQWTYQIYQEPFKNLKTGKYARMRGAHTNDVKQLTEAVQKIATESIVIWGKTPKFKLPIQKETWEAWWTEYWQATWIPEWEFVNTPPLVKLWYQLEKEPIVGAETFYVAGAANRETKLGKAGYVTDRGRQKVVSLTDTTNQKTALQAIHLALQDSGLEVNIVTASQYALGIIQAQPDKSESELVSQIIEQLIKKEKVYLAWVPAHKGIGGNEQVDKLVSRGIRKVLFLDGIDKAQEEHEKYHSNWRAMASEFNLPPIVAKEIVASCDKCQLKGEAIHGQVDCSPGIWQLACTHLEGKVILVAVHVASGYIEAEVIPAETGQETAYFLLKLAGRWPVKTIHTANGSNFTSATVKAACWWAGIKQEFGIPYNPQSQGVVASINKELKKIIGQVRDQAEHLKTAVQMAVFIHNFKRKGGIGEYSAGERIVDIIASDIQTKELQKQITKIQNFRVYYRDSRDPLWKGPAKLLWKGEGAVVIQDNSDIKVVPRRKAKIIRDYGKQMAGDDCVASRQDED

SEQ ID NO: 11 - protein, 625 aa, Artificial Sequence
  Mos1SEnv synthetic HIV envelope protein
MGNLWVTVYYGVPVWKDAKTTLFCASDAKAYEKEVHNVWATHACVPTDPNPQEIVLGNVTENFNMWKNDMVDQMHEDIISLWDASLEPCVKLTPLCVTLNCRNVRNVSSNGTYNIIHNETYKEMKNCSFNATTVVEDRKQKVHALFYRLDIVPLDENNSSEKSSENSSEYYRLINCNTSAITQACPKVSFDPIPIHYCAPAGYAILKCNNKTFNGTGPCNNVSTVQCTHGIKPVVSTQLLLNGSLAEEEIIIRSENLTNNAKTIIVHLNETVNITCTRPNNNTRKSIRIGPGQTFYATGDIIGDIRQAHCNLSRDGWNKTLQGVKKKLAEHFPNKTIKFAPHSGGDLEITTHTFNCRGEFFYCNTSNLFNESNIERNDSIITLPCRIKQIINMWQEVGRAIYAPPIAGNITCRSNITGLLLTRDGGSNNGVPNDTETFRPGGGDMRNNWRSELYKYKVVEVKPLGVAPTEAKRRVVEREKRAVGIGAVFLGILGAAGSTMGAASITLTVQARQLLSGIVQQQSNLLRAIEAQQHMLQLTVWGIKQLQTRVLAIERYLQDQQLLGLWGCSGKLICTTAVPWNTSWSNKSQTDIWDNMTWMQWDKEIGNYTGEIYRLLEESQNQQEK

SEQ ID NO: 12 - protein, 711 aa, Artificial Sequence
  Mos2SEnv synthetic HIV envelope protein
MRVRGMLRNWQQWWIWSSLGFWMLMIYSVMGNLWVTVYYGVPVWKDAKTTLFCASDAKAYEKEVHNVWATHACVPTDPNPQEIVLGNVTENFNMWKNDMVDQMHEDIISLWDASLEPCVKLTPLCVTLNCRNVRNVSSNGTYNIIHNETYKEMKNCSFNATTVVEDRKQKVHALFYRLDIVPLDENNSSEKSSENSSEYYRLINCNTSAITQACPKVSFDPIPIHYCAPAGYAILKCNNKTFNGTGPCNNVSTVQCTHGIKPVVSTQLLLNGSLAEEEIIIRSENLTNNAKTIIVHLNETVNITCTRPNNNTRKSIRIGPGQTFYATGDIIGDIRQAHCNLSRDGWNKTLQGVKKKLAEHFPNKTIKFAPHSGGDLEITTHTFNCRGEFFYCNTSNLFNESNIERNDSIITLPCRIKQIINMWQEVGRAIYAPPIAGNITCRSNITGLLLTRDGGSNNGVPNDTETFRPGGGDMRNNWRSELYKYKVVEVKPLGVAPTEAKRRVVEREKRAVGIGAVFLGILGAAGSTMGAASITLTVQARQLLSGIVQQQSNLLRAIEAQQHMLQLTVWGIKQLQTRVLAIERYLQDQQLLGLWGCSGKLICTTAVPWNTSWSNKSQTDIWDNMTWMQWDKEIGNYTGEIYRLLEESQNQQEKNEKDLLALDSWNNLWNWFSISKWLWYIKIFIMIVGGLIGLRIIFAVLSIVNRVRQGY

SEQ ID NO: 13 - protein, 30 aa, Artificial Sequence
  T4-fibritin "foldon" trimerization domain
GSGGYIPEAPRDGQAYVRKDGEWVLLSTFL

SEQ ID NO: 14 - protein, 32 aa, Artificial Sequence
  coiled-coil trimerization domain derived from GCN4
MKQIEDKIEEILSKIYHIENEIARIKKLIGEV